European Patent Specification EP 3 494 996 B1, published April 15, 2026. Title: ANTIBODY DRUG CONJUGATES (ADC) THAT BIND TO 158P1D7 PROTEINS. Applicant: AGENSYS, INC. SEATTLE GENETICS, INC. Application Divisional Application based on EP 13831502.3. The sequence listing filed with the application follows.

SEQUENCE LISTING (10 sequences)

SEQ ID NO: 1 - DNA, 2555 bp, Homo sapiens
  CDS (23)...(2548)
  misc_feature (1)...(2555): 158P1D7
tcggatttcatcacatgacaacatgaagctgtggattcatctcttttattcatctctccttgcctgtatatctttacactcccaaactccagtgctctcatccagaggctcttgtgattctctttgcaattgtgaggaaaaagatggcacaatgctaataaattgtgaagcaaaaggtatcaagatggtatctgaaataagtgtgccaccatcacgacctttccaactaagcttattaaataacggcttgacgatgcttcacacaaatgacttttctgggcttaccaatgctatttcaatacaccttggatttaacaatattgcagatattgagataggtgcatttaatggccttggcctcctgaaacaacttcatatcaatcacaattctttagaaattcttaaagaggatactttccatggactggaaaacctggaattcctgcaagcagataacaattttatcacagtgattgaaccaagtgcctttagcaagctcaacagactcaaagtgttaattttaaatgacaatgctattgagagtcttcctccaaacatcttccgatttgttcctttaacccatctagatcttcgtggaaatcaattacaaacattgccttatgttggttttctcgaacacattggccgaatattggatcttcagttggaggacaacaaatgggcctgcaattgtgacttattgcagttaaaaacttggttggagaacatgcctccacagtctataattggtgatgttgtctgcaacagccctccattttttaaaggaagtatactcagtagactaaagaaggaatctatttgccctactccaccagtgtatgaagaacatgaggatccttcaggatcattacatctggcagcaacatcttcaataaatgatagtcgcatgtcaactaagaccacgtccattctaaaactacccaccaaagcaccaggtttgataccttatattacaaagccatccactcaacttccaggaccttactgccctattccttgtaactgcaaagtcctatccccatcaggacttctaatacattgtcaggagcgcaacattgaaagcttatcagatctgagacctcctccgcaaaatcctagaaagctcattctagcgggaaatattattcacagtttaatgaagtctgatctagtggaatatttcactttggaaatgcttcacttgggaaacaatcgtattgaagttcttgaagaaggatcgtttatgaacctaacgagattacaaaaactctatctaaatggtaaccacctgaccaaattaagtaaaggcatgttccttggtctccataatcttgaatacttatatcttgaatacaatgccattaaggaaatactgccaggaacctttaatccaatgcctaaacttaaagtcctgtatttaaataacaacctcctccaagttttaccaccacatattttttcaggggttcctctaactaaggtaaatcttaaaacaaaccagtttacccatctacctgtaagtaatattttggatgatcttgatttactaacccagattgaccttgaggataacccctgggactgctcctgtgacctggttggactgcagcaatggatacaaaagttaagcaagaacacagtgacagatgacatcctctgcacttcccccgggcatctcgacaaaaaggaattgaaagccctaaatagtgaaattctctgtccaggtttagtaaataacccatccatgccaacacagactagttaccttatggtcaccactcctgcaacaacaacaaatacggctgatactattttacgatctcttacggacgctgtgccactgtctgttctaatattgggacttctgattatgttcatcactattgttttctgtgctgcagggatagtggttcttgttcttcaccgcaggagaagatacaaaaagaaacaagtagatgagcaaatgagagacaacagtcctgtgcatcttcagtacagcatgtatggccataaaaccactcatcacactactgaaagaccctctgcctcactctatgaacagcacatggtgagccccatggttcatgtctatagaagtccatcctttggtccaaagcatctggaagaggaagaagagaggaatgagaaagaaggaagtgatgcaaaacatctccaaagaagtcttttggaacaggaaaatcattcaccactcacagggtcaaatatgaaatacaaaaccacgaaccaatcaacagaatttttatccttccaagatgccagctcattgtacagaaacattttagaaaaagaaagggaacttcagcaactgggaatcacagaatacctaaggaaaaacattgctcagctccagcctgatatggaggcacattatcctggagcccacgaagagctgaagttaatggaaacattaatgtactcacgtccaaggaaggtattagtggaacagacaaaaaatgagtattttgaacttaaagctaatttacatgctgaacctgactatttagaagtcctggagcagcaaacatagatggaga

SEQ ID NO: 2 - protein, 841 aa, Homo sapiens
  misc_feature (1)...(842): 158P1D7
MKLWIHLFYSSLLACISLHSQTPVLSSRGSCDSLCNCEEKDGTMLINCEAKGIKMVSEISVPPSRPFQLSLLNNGLTMLHTNDFSGLTNAISIHLGFNNIADIEIGAFNGLGLLKQLHINHNSLEILKEDTFHGLENLEFLQADNNFITVIEPSAFSKLNRLKVLILNDNAIESLPPNIFRFVPLTHLDLRGNQLQTLPYVGFLEHIGRILDLQLEDNKWACNCDLLQLKTWLENMPPQSIIGDVVCNSPPFFKGSILSRLKKESICPTPPVYEEHEDPSGSLHLAATSSINDSRMSTKTTSILKLPTKAPGLIPYITKPSTQLPGPYCPIPCNCKVLSPSGLLIHCQERNIESLSDLRPPPQNPRKLILAGNIIHSLMKSDLVEYFTLEMLHLGNNRIEVLEEGSFMNLTRLQKLYLNGNHLTKLSKGMFLGLHNLEYLYLEYNAIKEILPGTFNPMPKLKVLYLNNNLLQVLPPHIFSGVPLTKVNLKTNQFTHLPVSNILDDLDLLTQIDLEDNPWDCSCDLVGLQQWIQKLSKNTVTDDILCTSPGHLDKKELKALNSEILCPGLVNNPSMPTQTSYLMVTTPATTTNTADTILRSLTDAVPLSVLILGLLIMFITIVFCAAGIVVLVLHRRRRYKKKQVDEQMRDNSPVHLQYSMYGHKTTHHTTERPSASLYEQHMVSPMVHVYRSPSFGPKHLEEEEERNEKEGSDAKHLQRSLLEQENHSPLTGSNMKYKTTNQSTEFLSFQDASSLYRNILEKERELQQLGITEYLRKNIAQLQPDMEAHYPGAHEELKLMETLMYSRPRKVLVEQTKNEYFELKANLHAEPDYLEVLEQQT

SEQ ID NO: 3 - DNA, 1341 bp, Homo sapiens
  CDS (1)...(1341)
  misc_feature (1)...(1341): Ha15-10ac12 heavy chain
  misc_feature (1)...(360): heavy chain variable region
  misc_feature (361)...(1341): heavy chain human IgG2 constant region
caggtgcagctggtggagtctgggggaggcgtggtccagcctgggaggtccctgagactctcctgtgcagcgtctggattcaccttcagtagctatggcatgcactgggtccgccaggctccaggcaaggggctggaatgggtggcagttatatggtatgatggaagtaatcaatattatgcagactccgtgaagggccgattcaccatctccagagacaattccaagaacacgctgtttctgcaaatgcacagcctgagagccgaggacacggctgtgtattactgtgcgagaggtctgacttctggacggtacggtatggacgtctggggccaagggaccacggtcaccgtctcctcagcctccaccaagggcccatcggtcttccccctggcgccctgctccaggagcacctccgagagcacagcggccctgggctgcctggtcaaggactacttccccgaaccggtgacggtgtcgtggaactcaggcgctctgaccagcggcgtgcacaccttcccagctgtcctacagtcctcaggactctactccctcagcagcgtggtgaccgtgccctccagcaacttcggcacccagacctacacctgcaacgtagatcacaagcccagcaacaccaaggtggacaagacagttgagcgcaaatgttgtgtcgagtgcccaccgtgcccagcaccacctgtggcaggaccgtcagtcttcctcttccccccaaaacccaaggacaccctcatgatctcccggacccctgaggtcacgtgcgtggtggtggacgtgagccacgaagaccccgaggtccagttcaactggtacgtggacggcgtggaggtgcataatgccaagacaaagccacgggaggagcagttcaacagcacgttccgtgtggtcagcgtcctcaccgttgtgcaccaggactggctgaacggcaaggagtacaagtgcaaggtctccaacaaaggcctcccagcccccatcgagaaaaccatctccaaaaccaaagggcagccccgagaaccacaggtgtacaccctgcccccatcccgggaggagatgaccaagaaccaggtcagcctgacctgcctggtcaaaggcttctaccccagcgacatcgccgtggagtgggagagcaatgggcagccggagaacaactacaagaccacacctcccatgctggactccgacggctccttcttcctttacagcaagctcaccgtggacaagagcaggtggcagcaggggaacgtcttctcatgctccgtgatgcatgaggctctgcacaaccactacacgcagaagagcctctccctgtctccgggtaaataa

SEQ ID NO: 4 - protein, 446 aa, Homo sapiens
  CHAIN (1)...(446): Ha15-10ac12 heavy chain
QVQLVESGGGVVQPGRSLRLSCAASGFTFSSYGMHWVRQAPGKGLEWVAVIWYDGSNQYYADSVKGRFTISRDNSKNTLFLQMHSLRAEDTAVYYCARGLTSGRYGMDVWGQGTTVTVSSASTKGPSVFPLAPCSRSTSESTAALGCLVKDYFPEPVTVSWNSGALTSGVHTFPAVLQSSGLYSLSSVVTVPSSNFGTQTYTCNVDHKPSNTKVDKTVERKCCVECPPCPAPPVAGPSVFLFPPKPKDTLMISRTPEVTCVVVDVSHEDPEVQFNWYVDGVEVHNAKTKPREEQFNSTFRVVSVLTVVHQDWLNGKEYKCKVSNKGLPAPIEKTISKTKGQPREPQVYTLPPSREEMTKNQVSLTCLVKGFYPSDIAVEWESNGQPENNYKTTPPMLDSDGSFFLYSKLTVDKSRWQQGNVFSCSVMHEALHNHYTQKSLSLSPGK

SEQ ID NO: 5 - DNA, 660 bp, Homo sapiens
  CDS (1)...(660)
  misc_feature (1)...(660): Ha15-10ac12 light chain
  misc_feature (1)...(339): light chain variable region
  misc_feature (340)...(660): human kappa constant region
gatattgtgatgactcagtctccactctccctgcccgtcacccctggagagccggcctccatctcctgcaggtctagtcagagcctcctgcttagtcatggattcaactatttggattggtacctgcagaagccagggcagtctccacaactcctgatctatttgggttctagtcgggcctccggggtccctgacaggttcagtggcagtggatcaggcacagattttacactgaaaatcagcagagtggaggctgaggatgttgggctttattactgcatgcaacccctacaaattccgtggacgttcggccaagggaccaaggtggaaatcaaacgaactgtggctgcaccatctgtcttcatcttcccgccatctgatgagcagttgaaatctggaactgcctctgttgtgtgcctgctgaataacttctatcccagagaggccaaagtacagtggaaggtggataacgccctccaatcgggtaactcccaggagagtgtcacagagcaggacagcaaggacagcacctacagcctcagcagcaccctgacgctgagcaaagcagactacgagaaacacaaagtctacgcctgcgaagtcacccatcagggcctgagctcgcccgtcacaaagagcttcaacaggggagagtgttag

SEQ ID NO: 6 - protein, 219 aa, Homo sapiens
  CHAIN (1)...(219): Ha15-10ac12 light chain
DIVMTQSPLSLPVTPGEPASISCRSSQSLLLSHGFNYLDWYLQKPGQSPQLLIYLGSSRASGVPDRFSGSGSGTDFTLKISRVEAEDVGLYYCMQPLQIPWTFGQGTKVEIKRTVAAPSVFIFPPSDEQLKSGTASVVCLLNNFYPREAKVQWKVDNALQSGNSQESVTEQDSKDSTYSLSSTLTLSKADYEKHKVYACEVTHQGLSSPVTKSFNRGEC

SEQ ID NO: 7 - protein, 446 aa, Homo sapiens; identical to SEQ ID NO: 4
  CHAIN (1)...(446): Ha15-10ac12 lheavy chain
  SITE (1)...(120): heavy chain variable region
  SITE (121)...(446): human IgG2 constant region

SEQ ID NO: 8 - protein, 219 aa, Homo sapiens; identical to SEQ ID NO: 6
  CHAIN (1)...(219): Ha15-10ac12 light chain
  SITE (1)...(113): light chain variable region
  SITE (114)...(219): human kappa constant region

SEQ ID NO: 9 - protein, 4 aa, Artificial Sequence
  synthetic construct
  misc_feature (1)...(4): peptidyl linker
GFLG

SEQ ID NO: 10 - protein, 100 aa, Homo sapiens
  DOMAIN (1)...(100): IGKV2D-28*01
DIVMTQSPLSLPVTPGEPASISCRSSQSLLHSNGYNYLDWYLQKPGQSPQLLIYLGSNRASGVPDRFSGSGSGTDFTLKISRVEAEDVGVYYCMQALQTP